European Patent Application EP 4 223 784 A2, published August 9, 2023. Title: Compositions and Methods for Modulating T-Cell Mediated Immune Response. Applicant: The Regents of the University of Colorado, A Body Corporate. Application EP. The sequence listing filed with the application follows.

SEQUENCE LISTING (123 sequences)

SEQ ID NO: 1 - protein, 326 aa, synthetic construct
  REGION 1..326: note = Fusion Protein
MRTEAQVPALQPPEPGLEGAMGHRTLVLPWVLLTLCVTAGTPEVWVQVRMEATELSSFTIRCGFLGSGSISLVTVSWGGPNGAGGTTLAVLHPERGIRQWAPARQARWETQSSISLILEGSGASSPCANTTFCCKFASFPEGSWEACGSLPPSSDPGLSAPPTPAPILRADLAGILGVSGVLLFGCVYLLHLLRRHKHRPAPRLQPSRTSPQAPRARAWAPSQASQAALHVPYATINTSCRPATLDTAHPHGGPSWWASLPTHAAHRPQGPAAWASTPIPARGSFVSVENGLYAQAGERPPHTGPGLTLFPDPRGPRAMEGPLGVR

SEQ ID NO: 2 - DNA, 1164 bp, synthetic construct
  misc_feature 1..1164: note = humanized antibody
  source 1..1164: mol_type = other DNA
gatcgacttagggcgattgatttagcggccgcgaattcgcccttctgcaaccggtgtacattccgacatcgtgatcacacagtctctgcaaccggtgtacattccgacattgagatgacacagtctccagccaccctgtctgtgactccaggagatagagtctctctttcctgcagggccagccagagtattagagactacttacactggtatcaacaaaaatcacatgagtctccaaggcttctcatcaaatatgtttcccaatccatttctgggatcccctccaggttcagtggcagtggatcagggtcagagttcactctcagtatcaacagtgtggaacctgaagatgttggagtatattactgtcaaaatggtcacagccttcctctcacgttcggctcggggacaaagttggaaataaaacgtacggtggcaagggcgaattcgtttaaacctgcaggactagtccctttagtgagggttaattctgagcttggcgtaatcatggtcatagctgtttcctgtgtgaaattgttatccgctcacaattccacacaacatacgagccggaagcataaagtgtaaagcctggggtgcctaatgagtgagctaactcacattaattgcgttgcgctcactgcccgctttccagtcgggaaacctgtcgtgccagctgcattaatgaatcggccaacgcgcggggagaggcggtttgcgtattgggcgctcttccgcttcctcgctcactgactcgctgcgctcggtcgttcggctgcggcgagcggtatcagctcactcaaaggcggtaatacggttatccacagaatcaggggataacgcaggaaagaacatgtgagcaaaaggccagcaaaaggccaggaaccgtaaaaaggccgcgttgctggcgtttttccataggctccgcccccctgacgagcatcacaaaaatcgacgctcaagtcagaggtggcgaaacccgacaggactataaagataccaggcgtttccccctgtaaagctccctcgtgcgctctcctgtttccgaccctgcccgctttaccgggataccctgtccgccctttttctcccttcggggaaagcgtgcgctttctcatagctcaacgctggtagattaatctctcaggttccggggttgtgtta

SEQ ID NO: 3 - protein, 110 aa, synthetic construct
  REGION 1..110: note = humanized antibody
DIEMTQSPATLSVTPGDRVSLSCRASQSIRDYLHWYQQKSHESPRLLIKYVSQSISGIPSRFSGSGSGSEFTLSINSVEPEDVGVYYCQNGHSLPLTFGSGTKLEIKRTV

SEQ ID NO: 4 - DNA, 383 bp, synthetic construct
  misc_feature 1..383: note = Humanized antibody
  source 1..383: mol_type = other DNA
gcaaccggtgtacattccgaggtgcaactgcagcagtcaggggctgaactggtgaggtctggggcctcagtgaagatgtcctgcaaggttaatgactacacatttaccaattacaatatgcactggttaaggcagacacctggccagggcctggaatggattggatatatttatcctggaaatggcgatactaactacaatcagaaattcaagggcaaggccacattgactgcagacacatcctccagcacagcctacatgcagatcatcagcctgacatctgaagaccctgcggtctatttctgtgcaagacagggaattcattactattacatcgatgtctggggcgcagggaccacggtcaccgtctcctcagggtcgac

SEQ ID NO: 5 - protein, 120 aa, synthetic construct
  REGION 1..120: note = Humanized antibody
EVQLQQSGAELVRSGASVKMSCKVNDYTFTNYNMHWLRQTPGQGLEWIGYIYPGNGDTNYNQKFKGKATLTADTSSSTAYMQIISLTSEDPAVYFCARQGIHYYYIDVWGAGTTVTVSSG

SEQ ID NO: 6 - protein, 10 aa, synthetic construct
  REGION 1..10: note = Humanized antibody
DYTFTNYNMH

SEQ ID NO: 7 - protein, 13 aa, synthetic construct
  REGION 1..13: note = Humanized antibody
YIYPGNGDTNYNQ

SEQ ID NO: 8 - protein, 10 aa, synthetic construct
  REGION 1..10: note = Humanized antibody
QGIHYYYIDV

SEQ ID NO: 9 - protein, 11 aa, synthetic construct
  REGION 1..11: note = Humanized antibody
RASQSIRDYLH

SEQ ID NO: 10 - protein, 7 aa, synthetic construct
  REGION 1..7: note = Humanized antibody
YVSQSIS

SEQ ID NO: 11 - protein, 9 aa, synthetic construct
  REGION 1..9: note = Humanized antibody
QNGHSLPLT

SEQ ID NO: 12 - protein, 15 aa, synthetic construct
  REGION 1..15: note = Synthetic tag
GLNDIFEAQKIEWHE

SEQ ID NO: 13 - protein, 26 aa, synthetic construct
  REGION 1..26: note = Synthetic tag
KRRWKKNFIAVSAANRFKKISSSGAL

SEQ ID NO: 14 - protein, 6 aa, synthetic construct
  REGION 1..6: note = synthetic tag
EEEEEE

SEQ ID NO: 15 - protein, 13 aa, synthetic construct
  REGION 1..13: note = Synthetic tag
GAPVPYPDPLEPR

SEQ ID NO: 16 - protein, 8 aa, synthetic construct
  REGION 1..8: note = synthetic tag
DYKDDDDK

SEQ ID NO: 17 - protein, 9 aa, synthetic construct
  REGION 1..9: note = Synthetic tag
YPYDVPDYA

SEQ ID NO: 18 - protein, 6 aa, synthetic construct
  REGION 1..6: note = Synthetic tag
HHHHHH

SEQ ID NO: 19 - protein, 10 aa, synthetic construct
  REGION 1..10: note = Synthetic tag
EQKLISEEDL

SEQ ID NO: 20 - protein, 15 aa, synthetic construct
  REGION 1..15: note = Synthetic tag
KETAAAKFERQHMDS

SEQ ID NO: 21 - protein, 38 aa, synthetic construct
  REGION 1..38: note = Synthetic tag
MDEKTTGWRGGHVVEGLAGELEQLRARLEHHPQGQREP

SEQ ID NO: 22 - protein, 13 aa, synthetic construct
  REGION 1..13: note = Synthetic tag
SLAELLNAGLGGS

SEQ ID NO: 23 - protein, 8 aa, synthetic construct
  REGION 1..8: note = Synthetic tag
TQDPSRVG

SEQ ID NO: 24 - protein, 8 aa, synthetic construct
  REGION 1..8: note = Synthetic tag
WSHPQFEK

SEQ ID NO: 25 - protein, 6 aa, synthetic construct
  REGION 1..6: note = Synthetic tag
CCPGCC

SEQ ID NO: 26 - protein, 14 aa, synthetic construct
  REGION 1..14: note = Synthetic tag
GKPIPNPLLGLDST

SEQ ID NO: 27 - protein, 11 aa, synthetic construct
  REGION 1..11: note = Synthetic tag
YTDIEMNRLGK

SEQ ID NO: 28 - protein, 8 aa, synthetic construct
  REGION 1..8: note = Synthetic tag
DLYDDDDK

SEQ ID NO: 29 - protein, 16 aa, synthetic construct
  REGION 1..16: note = Synthetic tag
TDKDMTITFTNKKDAE

SEQ ID NO: 30 - protein, 13 aa, synthetic construct
  REGION 1..13: note = Synthetic tag
AHIVMVDAYKPTK

SEQ ID NO: 31 - DNA, 25 bp, synthetic construct
  misc_feature 1..25: note = Recombinant sequence
  source 1..25: mol_type = other DNA
tgcacgtggcagctttgtctctgtt

SEQ ID NO: 32 - protein, 118 aa, synthetic construct
  REGION 1..118: note = Humanized antibody
QVQLQQSGAELAKPGASVKMSCKASGYTFTSDWMHWVKQRPGQGLEWIGYINPSTGYTEYNQKFKDKATLTADKSSSTAYMQLRSLTSEDSAVYYCARGSSGSWFAYWGQGTLVTVSA

SEQ ID NO: 33 - protein, 111 aa, synthetic construct
  REGION 1..111: note = Humanized antibody
DIVLTQSPASLAVSLGQRATISCRASQSVSTSSYSYMHWYQQKPGQPPKLLIKYASNLESGVPARFSGSGSGTDFTLNIHPVEEEDTATYYCQHSWEIPYTFGGGTKLEIK

SEQ ID NO: 34 - protein, 5 aa, synthetic construct
  REGION 1..5: note = Humanzed antibody
SDWMH

SEQ ID NO: 35 - protein, 17 aa, synthetic construct
  REGION 1..17: note = Humanized antibody
YINPSTGYTEYNQKFKD

SEQ ID NO: 36 - protein, 9 aa, synthetic construct
  REGION 1..9: note = Humanized antibody
GSSGSWFAY

SEQ ID NO: 37 - protein, 15 aa, synthetic construct
  REGION 1..15: note = Humanized antibody
RASQSVSTSSYSYMH

SEQ ID NO: 38 - protein, 7 aa, synthetic construct
  REGION 1..7: note = Humanized antibody
YASNLES

SEQ ID NO: 39 - protein, 9 aa, synthetic construct
  REGION 1..9: note = Humanized antibody
QHSWEIPYT

SEQ ID NO: 40 - protein, 112 aa, synthetic construct
  REGION 1..112: note = Humanized antibody
DVVMTQTPLTLSVTIGQPASISCKSSQSLLNSDGKTYLNWLLQRPGQSPKRLIYLVSKLDSGVPDRFTGSGSGTDFTLKISRVEAEDLGVYYCWQGTHFPRTFGGGTKLEIK

SEQ ID NO: 41 - protein, 16 aa, synthetic construct
  REGION 1..16: note = Humanized antibody
KSSQSLLNSDGKTYLN

SEQ ID NO: 42 - protein, 7 aa, synthetic construct
  REGION 1..7: note = Humanized antibody
LVSKLDS

SEQ ID NO: 43 - protein, 9 aa, synthetic construct
  REGION 1..9: note = Humanized antibody
WQGTHFPRT

SEQ ID NO: 44 - protein, 96 aa, synthetic construct
  REGION 1..96: note = Fusion protein
EATELSSFTIRCGFLGSGSISLVTVSWGGPNGAGGTTLAVLHPERGIRQWAPARQARWETQSSISLILEGSGASSPCANTTFCCKFASFPEGSWEA

SEQ ID NO: 45 - protein, 160 aa, synthetic construct
  REGION 1..160: note = Fusion protein
MRTEAQVPALQPPEPGLEGAMGHRTLVLPWVLLTLCVTAGTPEVWVQVRMEATELSSFTIRCGFLGSGSISLVTVSWGGPNGAGGTTLAVLHPERGIRQWAPARQARWETQSSISLILEGSGASSPCANTTFCCKFASFPEGSWEACGSLPPSSDPGLSA

SEQ ID NO: 46 - protein, 217 aa, synthetic construct
  REGION 1..217: note = Fusion Protein
APELLGGPSVFLFPPKPKDTLMISRTPEVTCVVVDVSHEDPEVKFNWYVDGVEVHNAKTKPREEQYNSTYRVVSVLTVLHQDWLNGKEYKCKVSNKALPAPIEKTISKAKGQPREPQVYTLPPSRDELTKNQVSLTCLVKGFYPSDIAVEWESNGQPENNYKTTPPVLDSDGSFFLYSKLTVDKSRWQQGNVFSCSVMHEALHNHYTQKSLSLSPGK

SEQ ID NO: 47 - protein, 216 aa, synthetic construct
  REGION 1..216: note = Fusion protein
APPVAGPSVFLFPPKPKDTLMISRTPEVTCVVVDVSHEDPEVQFNWYVDGVEVHNAKTKPREEQFNSTFRVVSVLTVVHQDWLNGKEYKCKVSNKGLPAPIEKTISKTKGQPREPQVYTLPPSREEMTKNQVSLTCLVKGFYPSDIAVEWESNGQPENNYKTTPPMLDSDGSFFLYSKLTVDKSRWQQGNVFSCSVMHEALHNHYTQKSLSLSPGK

SEQ ID NO: 48 - protein, 217 aa, synthetic construct
  REGION 1..217: note = Fusion protein
APELLGGPSVFLFPPKPKDTLMISRTPEVTCVVVDVSHEDPEVQFKWYVDGVEVHNAKTKPREEQYNSTFRVVSVLTVLHQDWLNGKEYKCKVSNKALPAPIEKTISKTKGQPREPQVYTLPPSREEMTKNQVSLTCLVKGFYPSDIAVEWESSGQPENNYNTTPPMLDSDGSFFLYSKLTVDKSRWQQGNIFSCSVMHEALHNRFTQKSLSLSPGK

SEQ ID NO: 49 - protein, 217 aa, synthetic construct
  REGION 1..217: note = Fusion protein
APEFLGGPSVFLFPPKPKDTLMISRTPEVTCVVVDVSQEDPEVQFNWYVDGVEVHNAKTKPREEQFNSTYRVVSVLTVLHQDWLNGKEYKCKVSNKGLPSSIEKTISKAKGQPREPQVYTLPPSQEEMTKNQVSLTCLVKGFYPSDIAVEWESNGQPENNYKTTPPVLDSDGSFFLYSRLTVDKSRWQEGNVFSCSVMHEALHNHYTQKSLSLSLGK

SEQ ID NO: 50 - protein, 218 aa, synthetic construct
  REGION 1..218: note = Fusion protein
IAELPPKVSVFVPPRDGFFGNPRKSKLICQATGFSPRQIQVSWLREGKQVGSGVTTDQVQAEAKESGPTTYKVTSTLTIKESDWLGQSMFTCRVDHRGLTFQQNASSMCVPDQDTAIRVFAIPPSFASIFLTKSTKLTCLVTDLTTYDSVTISWTRQNGEAVKTHTNISESHPNATFSAVGEASICEDDWNSGERFTCTVTHTDLPSPLKQTISRPKG

SEQ ID NO: 51 - DNA, 1467 bp, synthetic construct
  misc_feature 1..1467: note = Recombinant sequence
  source 1..1467: mol_type = other DNA
gccaccatgggatggagctgtatcatcctcttcttggtagcaacagctacaggtgtccacgaggtgcaactgcagcagtcaggggctgaactggtgaggtctggggcctcagtgaagatgtcctgcaaggttaatgactacacatttaccaattacaatatgcactggttaaggcagacacctggccagggcctggaatggattggatatatttatcctggaaatggcgatactaactacaatcagaaattcaagggcaaggccacattgactgcagacacatcctccagcacagcctacatgcagatcatcagcctgacatctgaagaccctgcggtctatttctgtgcaagacagggaattcattactattacatcgatgtctggggcgcagggaccacggtcaccgtctcctcagggggtggtggtggttctggtggtggtggttctggtggtggtggttctgacattgagatgacacagtctccagccaccctgtctgtgactccaggagatagagtctctctttcctgcagggccagccagagtattagagactacttacactggtatcaacaaaaatcacatgagtctccaaggcttctcatcaaatatgtttcccaatccatttctggcatcccctccaggttcagtggcagtggatcagggtcagagttcactctcagtatcaacagtgtggaacctgaagatgttggagtatattactgtcaaaatggtcacagccttcctctcacgttcggctcggggacaaagttggaaataaaacgtacggtgaccacgacgccagcgccgcgaccaccaacaccggcgcccaccatcgcgtcgcagcccctgtccctgcgcccagaggcgtgccggccagcggcggggggcgcagtgcacacgagggggctggacttcgcctgtgatatctacatctgggcgcccttggccgggacttgtggggtccttctcctgtcactggttatcaccaggagtaagaggagcaggctcctgcacagtgactacatgaacatgactccccgccgccccgggcccacccgcaagcattaccagccctatgccccaccacgcgacttcgcagcctatcgctccagagtgaagttcagcaggagcgcagacgcccccgcgtaccagcagggccagaaccagctctataacgagctcaatctaggacgaagagaggagtacgatgttttggacaagagacgtggccgggaccctgagatggggggaaagccgcagagaaggaagaaccctcaggaaggcctgtacaatgaactgcagaaagataagatggcggaggcctacagtgagattgggatgaaaggcgagcgccggaggggcaaggggcacgatggcctttaccagggtctcagtacagccaccaaggacacctacgacgcccttcacatgcaggccctgccccctcgcaaaccggtttaa

SEQ ID NO: 52 - protein, 394 aa, synthetic construct
  REGION 1..394: note = fusion protein
MRTEAQVPALQPPEPGLEGAMGHRTLVLPWVLLTLCVTAGTPEVWVQVRMEATELSSFTIRCGFLGSGSISLVTVSWGGPNGAGGTTLAVLHPERGIRQWAPARQARWETQSSISLILEGSGASSPCANTTFCCKFASFPEGSWEACGSLPPSSDPGLSARSPRGPTIKPCPPCKCPAPNLLGGPSVFIFPPKIKDVLMISLSPIVTCVVVDVSEDDPDVQISWFVNNVEVHTAQTQTHREDYNSTLRVVSALPIQHQDWMSGKEFKCKVNNKDLPAPIERTISKPKGSVRAPQVYVLPPPEEEMTKKQVTLTCMVTDFMPEDIYVEWTNNGKTELNYKNTEPVLDSDGSYFMYSKLRVEKKNWVERNSYSCSVVHEGLHNHHTTKSFSRTPGK

SEQ ID NO: 53 - protein, 17 aa, Homo sapiens
AVLHPERGIRQWAPARQ

SEQ ID NO: 54 - protein, 20 aa, Homo sapiens
AVLHPERGIRQWAPARQARW

SEQ ID NO: 55 - protein, 25 aa, Homo sapiens
AVLHPERGIRQWAPARQARWETQSS

SEQ ID NO: 56 - protein, 27 aa, Homo sapiens
AVLHPERGIRQWAPARQARWETQSSIS

SEQ ID NO: 57 - protein, 28 aa, Homo sapiens
AVLHPERGIRQWAPARQARWETQSSISL

SEQ ID NO: 58 - DNA, 25 bp, synthetic construct
  misc_feature 1..25: note = Recombinant sequence
  source 1..25: mol_type = other DNA
acgtggcagctttgtctctgttgag

SEQ ID NO: 59 - DNA, 25 bp, synthetic construct
  misc_feature 1..25: note = Recombinant Sequence
  source 1..25: mol_type = other DNA
tggcagctttgtctctgttgagaat

SEQ ID NO: 60 - DNA, 25 bp, synthetic construct
  misc_feature 1..25: note = recombinant sequence
  source 1..25: mol_type = other DNA
gctttgtctctgttgagaatggact

SEQ ID NO: 61 - protein, 100 aa, Homo sapiens
VQVRMEATELSSFTIRCGFLGSGSISLVTVSWGGPNGAGGTTLAVLHPERGIRQWAPARQARWETQSSISLILEGSGASSPCANTTFCCKFASFPEGSWE

SEQ ID NO: 62 - protein, 116 aa, Homo sapiens
VQVLPEVRGQLGGTVELPCHLLPPVPGLYISLVTWQRPDAPANHQNVAAFHPKMGPSFPSPKPGSERLSFVSAKQSTGQDTEAELQDATLALHGLTVEDEGNYTCEFATFPKGSVR

SEQ ID NO: 63 - protein, 105 aa, Homo sapiens
VQAPTQVPGFLGDSVTLPCYLQVPNMEVTHVSQLTWARHGESGSMAVFHQTQGPSYSESKKRLEFVAARLGAELRNASLRMFGLRVEDEGNYTCLFVTFPQGSRS

SEQ ID NO: 64 - protein, 93 aa, Homo sapiens
IETTGNISAEKGGSIILQCHLSSTTAQVTQVNWEQQDQLLAICNADLGWHISPSFKDRVAPGPGLGLTLQSLTVNDTGEYFCIYHTYPDGTYT

SEQ ID NO: 65 - protein, 103 aa, Homo sapiens
VNTEENVYATLGSDVNLTCQTQTVGFFVQMQWSKVTNKIDLIAVYHPQYGFYCATGRPCESLVTFTETPENGSKWTLHLRNMSCSVSGRYECMLVLYPEGIQT

SEQ ID NO: 66 - protein, 103 aa, Homo sapiens
VQVNDSMYGFIGTDVVLHCSFANPLPSVKITQVTWQKSTNGSKQNVAIYNPSMGVSVLAPYRERVEFLRPSFTDGTIRLSRLELEDEGVYICEFATFPTGNRE

SEQ ID NO: 67 - protein, 100 aa, Homo sapiens
IIVEPHVTAVWGKNVSLKCLIEVNETITQISWEKIHGKSSQTVAVHHPQYGFSVQGEYQGRVLFKNYSLNDATITLHNIGFSDSGKYICKAVTFPLGNAQ

SEQ ID NO: 68 - protein, 105 aa, Homo sapiens
LETSDVVTVVLGQDAKLPCFYRGDSGEQVGQVAWARVDAGEGAQELALLHSKYGLHVSPAYEGRVEQPPPPRNPLDGSVLLRNAVQADEGEYECRVSTFPAGSFQ

SEQ ID NO: 69 - protein, 102 aa, Homo sapiens
EEVLWHTSVPFAENMSLECVYPSMGILTQVEWFKIGTQQDSIAIFSPTHGMVIRKPYAERVYFLNSTMASNNMTLFFRNASEDDVGYYSCSLYTTYPQGTWQ

SEQ ID NO: 70 - protein, 10 aa, Homo sapiens
EAQVPALQPP

SEQ ID NO: 71 - protein, 26 aa, Homo sapiens
VLPWVLLTLCVTAGTPEVWVQVRMEA

SEQ ID NO: 72 - protein, 32 aa, Homo sapiens
PWVLLTLCVTAGTPEVWQVRMEATELSSFTIR

SEQ ID NO: 73 - protein, 7 aa, Homo sapiens
LCVTAGT

SEQ ID NO: 74 - protein, 10 aa, Homo sapiens
VTVSWGGPNG

SEQ ID NO: 75 - protein, 17 aa, Homo sapiens
AVLHPERGIRQWAPARQ

SEQ ID NO: 76 - protein, 20 aa, Homo sapiens
AVLHPERGIRQWAPARQARW

SEQ ID NO: 77 - protein, 25 aa, Homo sapiens
AVLHPERGIRQWAPARQARWETQSS

SEQ ID NO: 78 - protein, 27 aa, Homo sapiens
AVLHPERGIRQWAPARQARWETQSSIS

SEQ ID NO: 79 - protein, 28 aa, Homo sapiens
AVLHPERGIRQWAPARQARWETQSSISL

SEQ ID NO: 80 - protein, 9 aa, Homo sapiens
LSARSPRGP

SEQ ID NO: 81 - protein, 11 aa, Homo sapiens
CKCPAPNLLGG

SEQ ID NO: 82 - protein, 10 aa, Homo sapiens
VFIFPPKIKD

SEQ ID NO: 83 - protein, 12 aa, Homo sapiens
VFIFPPKIKDVL

SEQ ID NO: 84 - protein, 9 aa, Homo sapiens
FIFPPKIKD

SEQ ID NO: 85 - protein, 11 aa, Homo sapiens
FIFPPKIKDVL

SEQ ID NO: 86 - protein, 12 aa, Homo sapiens
FIFPPKIKDVLM

SEQ ID NO: 87 - protein, 8 aa, Homo sapiens
IFPPKIKD

SEQ ID NO: 88 - protein, 7 aa, Homo sapiens
FPPKIKD

SEQ ID NO: 89 - protein, 10 aa, Homo sapiens
FPPKIKDVLM

SEQ ID NO: 90 - protein, 9 aa, Homo sapiens
PPKIKDVLM

SEQ ID NO: 91 - protein, 7 aa, Homo sapiens
PKIKDVL

SEQ ID NO: 92 - protein, 9 aa, Homo sapiens
MISLSPIVT

SEQ ID NO: 93 - protein, 8 aa, Homo sapiens
ISLSPIVT

SEQ ID NO: 94 - protein, 9 aa, Homo sapiens
VSEDDPDVQ

SEQ ID NO: 95 - protein, 14 aa, Homo sapiens
FVNNVEVHTAQTQT

SEQ ID NO: 96 - protein, 23 aa, Homo sapiens
LRVVSALPIQHQDWMSGKEFKCK

SEQ ID NO: 97 - protein, 13 aa, Homo sapiens
RVVSALPIQHQDW

SEQ ID NO: 98 - protein, 18 aa, Homo sapiens
RVVSALPIQHQDWMSGKE

SEQ ID NO: 99 - protein, 11 aa, Homo sapiens
VSALPIQHQDW

SEQ ID NO: 100 - protein, 7 aa, Homo sapiens
PIQHQDW

SEQ ID NO: 101 - protein, 12 aa, Homo sapiens
PIQHQDWMSGKE

SEQ ID NO: 102 - protein, 15 aa, Homo sapiens
FKCKVNNKDLPAPIE

SEQ ID NO: 103 - protein, 14 aa, Homo sapiens
LPAPIERTISKPKG

SEQ ID NO: 104 - protein, 15 aa, Homo sapiens
RTISKPKGSVRAPQV

SEQ ID NO: 105 - protein, 24 aa, Homo sapiens
GSVRAPQVYVLPPPEEEMTKKQVT

SEQ ID NO: 106 - protein, 8 aa, Homo sapiens
YVLPPPEE

SEQ ID NO: 107 - protein, 8 aa, Homo sapiens
KKQVTLTC

SEQ ID NO: 108 - protein, 9 aa, Homo sapiens
VTDFMPEDI

SEQ ID NO: 109 - protein, 10 aa, Homo sapiens
VTDFMPEDIY

SEQ ID NO: 110 - protein, 8 aa, Homo sapiens
DFMPEDIY

SEQ ID NO: 111 - protein, 10 aa, Homo sapiens
FMPEDIYVEW

SEQ ID NO: 112 - protein, 13 aa, Homo sapiens
IYVEWTNNGKTEL

SEQ ID NO: 113 - protein, 12 aa, Homo sapiens
YVEWTNNGKTEL

SEQ ID NO: 114 - protein, 11 aa, Homo sapiens
VEWTNNGKTEL

SEQ ID NO: 115 - protein, 10 aa, Homo sapiens
EWTNNGKTEL

SEQ ID NO: 116 - protein, 9 aa, Homo sapiens
NYKNTEPVL

SEQ ID NO: 117 - protein, 7 aa, Homo sapiens
KNTEPVL

SEQ ID NO: 118 - protein, 20 aa, Homo sapiens
TEPVLDSDGSYFMYSKLRVE

SEQ ID NO: 119 - protein, 7 aa, Homo sapiens
DSDGSYF

SEQ ID NO: 120 - protein, 16 aa, Homo sapiens
RVEKKNWVERNSYSCS

SEQ ID NO: 121 - protein, 8 aa, Homo sapiens
SVVHEGLH

SEQ ID NO: 122 - protein, 8 aa, synthetic construct
DSDGSYFM

SEQ ID NO: 123 - DNA, 25 bp, synthetic construct
  misc_feature 1..25: note = recombinant sequence
  source 1..25: mol_type = other DNA
tgcacgtggcagctttgtctctgtt